European Patent Application EP 4 484 566 A1, published January 1, 2025. Title: ATP production from electricity with a new-to-nature electrobiological module. Applicant: Max-Planck-Gesellschaft fuer Foerderung der Wissenschaften e.V. Application EP. The sequence listing filed with the application follows.

SEQUENCE LISTING (14 sequences)

SEQ ID NO: 1 - DNA, 25 bp, synthetic construct
  source 1..25: mol_type = other DNA
aatgacgcaaacatcgccgatgtcg

SEQ ID NO: 2 - DNA, 27 bp, synthetic construct
  source 1..27: mol_type = other DNA
tcaacggatattgagcgcttccaccat

SEQ ID NO: 3 - DNA, 27 bp, synthetic construct
  source 1..27: mol_type = other DNA
atggtggaagcgctcaatatccgttga

SEQ ID NO: 4 - DNA, 25 bp, synthetic construct
  source 1..25: mol_type = other DNA
cgacatcggcgatgtttgcgtcatt

SEQ ID NO: 5 - DNA, 18 bp, synthetic construct
  source 1..18: mol_type = other DNA
cggttcctggccttttgc

SEQ ID NO: 6 - DNA, 23 bp, synthetic construct
  source 1..23: mol_type = other DNA
gataggtgcctcactgattaagc

SEQ ID NO: 7 - DNA, 19 bp, synthetic construct
  source 1..19: mol_type = other DNA
gatcttaaggctagagtac

SEQ ID NO: 8 - DNA, 18 bp, synthetic construct
  source 1..18: mol_type = other DNA
caaaaaacccctcaagac

SEQ ID NO: 9 - DNA, 1539 bp, synthetic construct
  source 1..1539: mol_type = other DNA
atgaatgacgcaaacatcgccgatgtcgtgacgaaggtcctcggcgaatatggcgcgcctggtgcggtgtcggtcgcggcgctgaccgccaagagccccgacgggaaaagcaactcgtccgccgatgcggatgtggtcgcccggatggtggccaaggcgatccgcgaccacgccggaactgcgcagccgtccggtaacgccgcgacgtcgtcggcggcggtcagcgatggcgtgttcgagaccatggatgccgcggtcgaggccgctgctctggcgcagcagcaatacctgctttgctcgatgtccgaccgcgcgcgcttcgtgcagggaatccgcgacgtcatcttgaatcaggatacgctcgaaaagatgtcccgcatggcggtcgaagaaaccggcatgggcaattacgagcataagctgatcaagaaccggctagccggcgaaaagaccccgggcatcgaagatctcaccaccgacgctttcagcggcgacaacggtctgacgctggtggaatactcgccgttcggggtgatcggcgcgatcacgccgaccaccaatccgacggaaaccatcgtctgcaattcgatcggaatgctggcggccggcaacagcgtggtgttcagcccgcatggacgcgcccggcaggtgtcgctgctgctggtccgcctgatcaaccagaagctggcagcgctcggcgcgccggaaaacctggtggtgaccgtggagaagccctcgagagagaacacccttgccatgatggcgcatcccaaggtgcggatgctggttgccaccggcggccccgccctcgtcaaggcggtgctgtcgaccggcaagaaggcgatcggcgccggcgccggcaatccgcccgtcgtggtcgacgaaaccgccaacatcgaaaaagccgcctgcgacatcgtcaatggctgcagcttcgacaacaacctgccctgcgtcgccgagaaggagatcatcgcagtcgcccagatcgccgattacctgatcttcaacttgaagaagaacggcgcctacgagatcaaggatccggcggttctgcagcaactgcaggacctggtgctgaccgccaagggcgggccacagaccaaatgcgtcggcaagagtgcggtgtggctgctgtcgcagatcggcatcagcgtcgacgccagcatcaagatcatcctgatggaagtgccgcgggaacatcccttcgtgcaggaagaactgatgatgccgatcctgccgctggtccgggtcgaaaccgtggatgatgcgatcgacctcgccatcgaggtggagcacgacaatcgccacaccgcgatcatgcattccaccgatgtgcgcaagctcaccaagatggccaagctgatccagaccacgatcttcgtgaagaacggcccgtcttatgcggggctcggcgccggcggcgagggatattccaccttcaccatcgcgggtcccacgggcgagggcctgacctcggcgaagtcgttcgcgcgccgccgcaaatgcgtgatggtggaagcgctcaatatccgttga

SEQ ID NO: 10 - DNA, 6886 bp, synthetic construct
  source 1..6886: mol_type = other DNA
tggcgaatgggacgcgccctgtagcggcgcattaagcgcggcgggtgtggtggttacgcgcagcgtgaccgctacacttgccagcgccctagcgcccgctcctttcgctttcttcccttcctttctcgccacgttcgccggctttccccgtcaagctctaaatcgggggctccctttagggttccgatttagtgctttacggcacctcgaccccaaaaaacttgattagggtgatggttcacgtagtgggccatcgccctgatagacggtttttcgccctttgacgttggagtccacgttctttaatagtggactcttgttccaaactggaacaacactcaaccctatctcggtctattcttttgatttataagggattttgccgatttcggcctattggttaaaaaatgagctgatttaacaaaaatttaacgcgaattttaacaaaatattaacgtttacaatttcaggtggcacttttcggggaaatgtgcgcggaacccctatttgtttatttttctaaatacattcaaatatgtatccgctcatgaattaattcttagaaaaactcatcgagcatcaaatgaaactgcaatttattcatatcaggattatcaataccatatttttgaaaaagccgtttctgtaatgaaggagaaaactcaccgaggcagttccataggatggcaagatcctggtatcggtctgcgattccgactcgtccaacatcaatacaacctattaatttcccctcgtcaaaaataaggttatcaagtgagaaatcaccatgagtgacgactgaatccggtgagaatggcaaaagtttatgcatttctttccagacttgttcaacaggccagccattacgctcgtcatcaaaatcactcgcatcaaccaaaccgttattcattcgtgattgcgcctgagcgagacgaaatacgcgatcgctgttaaaaggacaattacaaacaggaatcgaatgcaaccggcgcaggaacactgccagcgcatcaacaatattttcacctgaatcaggatattcttctaatacctggaatgctgttttcccggggatcgcagtggtgagtaaccatgcatcatcaggagtacggataaaatgcttgatggtcggaagaggcataaattccgtcagccagtttagtctgaccatctcatctgtaacatcattggcaacgctacctttgccatgtttcagaaacaactctggcgcatcgggcttcccatacaatcgatagattgtcgcacctgattgcccgacattatcgcgagcccatttatacccatataaatcagcatccatgttggaatttaatcgcggcctagagcaagacgtttcccgttgaatatggctcataacaccccttgtattactgtttatgtaagcagacagttttattgttcatgaccaaaatcccttaacgtgagttttcgttccactgagcgtcagaccccgtagaaaagatcaaaggatcttcttgagatcctttttttctgcgcgtaatctgctgcttgcaaacaaaaaaaccaccgctaccagcggtggtttgtttgccggatcaagagctaccaactctttttccgaaggtaactggcttcagcagagcgcagataccaaatactgtccttctagtgtagccgtagttaggccaccacttcaagaactctgtagcaccgcctacatacctcgctctgctaatcctgttaccagtggctgctgccagtggcgataagtcgtgtcttaccgggttggactcaagacgatagttaccggataaggcgcagcggtcgggctgaacggggggttcgtgcacacagcccagcttggagcgaacgacctacaccgaactgagatacctacagcgtgagctatgagaaagcgccacgcttcccgaagggagaaaggcggacaggtatccggtaagcggcagggtcggaacaggagagcgcacgagggagcttccagggggaaacgcctggtatctttatagtcctgtcgggtttcgccacctctgacttgagcgtcgatttttgtgatgctcgtcaggggggcggagcctatggaaaaacgccagcaacgcggcctttttacggttcctggccttttgctggccttttgctcacatgttctttcctgcgttatcccctgattctgtggataaccgtattaccgcctttgagtgagctgataccgctcgccgcagccgaacgaccgagcgcagcgagtcagtgagcgaggaagcggaagagcgcctgatgcggtattttctccttacgcatctgtgcggtatttcacaccgcatatatggtgcactctcagtacaatctgctctgatgccgcatagttaagccagtatacactccgctatcgctacgtgactgggtcatggctgcgccccgacacccgccaacacccgctgacgcgccctgacgggcttgtctgctcccggcatccgcttacagacaagctgtgaccgtctccgggagctgcatgtgtcagaggttttcaccgtcatcaccgaaacgcgcgaggcagctgcggtaaagctcatcagcgtggtcgtgaagcgattcacagatgtctgcctgttcatccgcgtccagctcgttgagtttctccagaagcgttaatgtctggcttctgataaagcgggccatgttaagggcggttttttcctgtttggtcactgatgcctccgtgtaagggggatttctgttcatgggggtaatgataccgatgaaacgagagaggatgctcacgatacgggttactgatgatgaacatgcccggttactggaacgttgtgagggtaaacaactggcggtatggatgcggcgggaccagagaaaaatcactcagggtcaatgccagcgcttcgttaatacagatgtaggtgttccacagggtagccagcagcatcctgcgatgcagatccggaacataatggtgcagggcgctgacttccgcgtttccagactttacgaaacacggaaaccgaagaccattcatgttgttgctcaggtcgcagacgttttgcagcagcagtcgcttcacgttcgctcgcgtatcggtgattcattctgctaaccagtaaggcaaccccgccagcctagccgggtcctcaacgacaggagcacgatcatgcgcacccgtggggccgccatgccggcgataatggcctgcttctcgccgaaacgtttggtggcgggaccagtgacgaaggcttgagcgagggcgtgcaagattccgaataccgcaagcgacaggccgatcatcgtcgcgctccagcgaaagcggtcctcgccgaaaatgacccagagcgctgccggcacctgtcctacgagttgcatgataaagaagacagtcataagtgcggcgacgatagtcatgccccgcgcccaccggaaggagctgactgggttgaaggctctcaagggcatcggtcgagatcccggtgcctaatgagtgagctaacttacattaattgcgttgcgctcactgcccgctttccagtcgggaaacctgtcgtgccagctgcattaatgaatcggccaacgcgcggggagaggcggtttgcgtattgggcgccagggtggtttttcttttcaccagtgagacgggcaacagctgattgcccttcaccgcctggccctgagagagttgcagcaagcggtccacgctggtttgccccagcaggcgaaaatcctgtttgatggtggttaacggcgggatataacatgagctgtcttcggtatcgtcgtatcccactaccgagatatccgcaccaacgcgcagcccggactcggtaatggcgcgcattgcgcccagcgccatctgatcgttggcaaccagcatcgcagtgggaacgatgccctcattcagcatttgcatggtttgttgaaaaccggacatggcactccagtcgccttcccgttccgctatcggctgaatttgattgcgagtgagatatttatgccagccagccagacgcagacgcgccgagacagaacttaatgggcccgctaacagcgcgatttgctggtgacccaatgcgaccagatgctccacgcccagtcgcgtaccgtcttcatgggagaaaataatactgttgatgggtgtctggtcagagacatcaagaaataacgccggaacattagtgcaggcagcttccacagcaatggcatcctggtcatccagcggatagttaatgatcagcccactgacgcgttgcgcgagaagattgtgcaccgccgctttacaggcttcgacgccgcttcgttctaccatcgacaccaccacgctggcacccagttgatcggcgcgagatttaatcgccgcgacaatttgcgacggcgcgtgcagggccagactggaggtggcaacgccaatcagcaacgactgtttgcccgccagttgttgtgccacgcggttgggaatgtaattcagctccgccatcgccgcttccactttttcccgcgttttcgcagaaacgtggctggcctggttcaccacgcgggaaacggtctgataagagacaccggcatactctgcgacatcgtataacgttactggtttcacattcaccaccctgaattgactctcttccgggcgctatcatgccataccgcgaaaggttttgcgccattcgatggtgtccgggatctcgacgctctcccttatgcgactcctgcattaggaagcagcccagtagtaggttgaggccgttgagcaccgccgccgcaaggaatggtgcatgcaaggagatggcgcccaacagtcccccggccacggggcctgccaccatacccacgccgaaacaagcgctcatgagcccgaagtggcgagcccgatcttccccatcggtgatgtcggcgatataggcgccagcaaccgcacctgtggcgccggtgatgccggccacgatgcgtccggcgtagaggatcgagatctcgatcccgcgaaattaatacgactcactataggggaattgtgagcggataacaattcccctctagaaataattttgtttaactttaagaaggagatataccatgggcagcagccatcatcatcatcatcacagcagcggcctggtgccgcgcggcagccatatggctagcatgactggtggacagcaaatgggtcgcggatccgaattcaatgacgcaaacatcgccgatgtcgtgacgaaggtcctcggcgaatatggcgcgcctggtgcggtgtcggtcgcggcgctgaccgccaagagccccgacgggaaaagcaactcgtccgccgatgcggatgtggtcgcccggatggtggccaaggcgatccgcgaccacgccggaactgcgcagccgtccggtaacgccgcgacgtcgtcggcggcggtcagcgatggcgtgttcgagaccatggatgccgcggtcgaggccgctgctctggcgcagcagcaatacctgctttgctcgatgtccgaccgcgcgcgcttcgtgcagggaatccgcgacgtcatcttgaatcaggatacgctcgaaaagatgtcccgcatggcggtcgaagaaaccggcatgggcaattacgagcataagctgatcaagaaccggctagccggcgaaaagaccccgggcatcgaagatctcaccaccgacgctttcagcggcgacaacggtctgacgctggtggaatactcgccgttcggggtgatcggcgcgatcacgccgaccaccaatccgacggaaaccatcgtctgcaattcgatcggaatgctggcggccggcaacagcgtggtgttcagcccgcatggacgcgcccggcaggtgtcgctgctgctggtccgcctgatcaaccagaagctggcagcgctcggcgcgccggaaaacctggtggtgaccgtggagaagccctcgagagagaacacccttgccatgatggcgcatcccaaggtgcggatgctggttgccaccggcggccccgccctcgtcaaggcggtgctgtcgaccggcaagaaggcgatcggcgccggcgccggcaatccgcccgtcgtggtcgacgaaaccgccaacatcgaaaaagccgcctgcgacatcgtcaatggctgcagcttcgacaacaacctgccctgcgtcgccgagaaggagatcatcgcagtcgcccagatcgccgattacctgatcttcaacttgaagaagaacggcgcctacgagatcaaggatccggcggttctgcagcaactgcaggacctggtgctgaccgccaagggcgggccacagaccaaatgcgtcggcaagagtgcggtgtggctgctgtcgcagatcggcatcagcgtcgacgccagcatcaagatcatcctgatggaagtgccgcgggaacatcccttcgtgcaggaagaactgatgatgccgatcctgccgctggtccgggtcgaaaccgtggatgatgcgatcgacctcgccatcgaggtggagcacgacaatcgccacaccgcgatcatgcattccaccgatgtgcgcaagctcaccaagatggccaagctgatccagaccacgatcttcgtgaagaacggcccgtcttatgcggggctcggcgccggcggcgagggatattccaccttcaccatcgcgggtcccacgggcgagggcctgacctcggcgaagtcgttcgcgcgccgccgcaaatgcgtgatggtggaagcgctcaatatccgttgagcggccgcactcgagcaccaccaccaccaccactgagatccggctgctaacaaagcccgaaaggaagctgagttggctgctgccaccgctgagcaataactagcataaccccttggggcctctaaacgggtcttgaggggttttttgctgaaaggaggaactatatccggat

SEQ ID NO: 11 - DNA, 7184 bp, synthetic construct
  source 1..7184: mol_type = other DNA
agcccagtagtaggttgaggccgttgagcaccgccgccgcaaggaatggtgcatgcaaggagatggcgcccaacagtcccccggccacggggcctgccaccatacccacgccgaaacaagcgctcatgagcccgaagtggcgagcccgatcttccccatcggtgatgtcggcgatataggcgccagcaaccgcacctgtggcgccggtgatgccggccacgatgcgtccggcgtagaggatcgagatctcgatcccgcgaaattaatacgactcactataggggaattgtgagcggataacaattcccctctagaaataattttgtttaactttaagaaggagatataccatggcgtggagccacccgcagttcgagaagggacatatgaatgacgcaaacatcgccgatgtcgtgacgaaggtcctcggcgaatatggcgcgcctggtgcggtgtcggtcgcggcgctgaccgccaagagccccgacgggaaaagcaactcgtccgccgatgcggatgtggtcgcccggatggtggccaaggcgatccgcgaccacgccggaactgcgcagccgtccggtaacgccgcgacgtcgtcggcggcggtcagcgatggcgtgttcgagaccatggatgccgcggtcgaggccgctgctctggcgcagcagcaatacctgctttgctcgatgtccgaccgcgcgcgcttcgtgcagggaatccgcgacgtcatcttgaatcaggatacgctcgaaaagatgtcccgcatggcggtcgaagaaaccggcatgggcaattacgagcataagctgatcaagaaccggctagccggcgaaaagaccccgggcatcgaagatctcaccaccgacgctttcagcggcgacaacggtctgacgctggtggaatactcgccgttcggggtgatcggcgcgatcacgccgaccaccaatccgacggaaaccatcgtctgcaattcgatcggaatgctggcggccggcaacagcgtggtgttcagcccgcatggacgcgcccggcaggtgtcgctgctgctggtccgcctgatcaaccagaagctggcagcgctcggcgcgccggaaaacctggtggtgaccgtggagaagccctcgagagagaacacccttgccatgatggcgcatcccaaggtgcggatgctggttgccaccggcggccccgccctcgtcaaggcggtgctgtcgaccggcaagaaggcgatcggcgccggcgccggcaatccgcccgtcgtggtcgacgaaaccgccaacatcgaaaaagccgcctgcgacatcgtcaatggctgcagcttcgacaacaacctgccctgcgtcgccgagaaggagatcatcgcagtcgcccagatcgccgattacctgatcttcaacttgaagaagaacggcgcctacgagatcaaggatccggcggttctgcagcaactgcaggacctggtgctgaccgccaagggcgggccacagaccaaatgcgtcggcaagagtgcggtgtggctgctgtcgcagatcggcatcagcgtcgacgccagcatcaagatcatcctgatggaagtgccgcgggaacatcccttcgtgcaggaagaactgatgatgccgatcctgccgctggtccgggtcgaaaccgtggatgatgcgatcgacctcgccatcgaggtggagcacgacaatcgccacaccgcgatcatgcattccaccgatgtgcgcaagctcaccaagatggccaagctgatccagaccacgatcttcgtgaagaacggcccgtcttatgcggggctcggcgccggcggcgagggatattccaccttcaccatcgcgggtcccacgggcgagggcctgacctcggcgaagtcgttcgcgcgccgccgcaaatgcgtgatggtggaagcgctcaatatccgttgaattcataatctttctagaagatctcctacaatattctcagctgccatggaaaatcgatgttcttcttttattctctcaagattttcaggctgtatattaaaacttatattaagaactatgctaaccacctcatcaggaaccgttgtaggtggcgtgggttttcttggcaatcgactctcatgaaaactacgagctaaatattcaatatgttcctcttgaccaactttattctgcattttttttgaacgaggtttagagcaagcttatcgatgataagctgtcaaacatgagaattcttgaagacgaaagggcctcgtgatacgcctatttttataggttaatgtcatgataataatggtttcttagacgtcaggtggcacttttcggggaaatgtgcgcggaacccctatttgtttatttttctaaatacattcaaatatgtatccgctcatgagacaataaccctgataaatgcttcaataatattgaaaaaggaagagtatgagtattcaacatttccgtgtcgcccttattcccttttttgcggcattttgccttcctgtttttgctcacccagaaacgctggtgaaagtaaaagatgctgaagatcagttgggtgcacgagtgggttacatcgaactggatctcaacagcggtaagatccttgagagttttcgccccgaagaacgttttccaatgatgagcacttttaaagttctgctatgtggcgcggtattatcccgtgttgacgccgggcaagagcaactcggtcgccgcatacactattctcagaatgacttggttgagtactcaccagtcacagaaaagcatcttacggatggcatgacagtaagagaattatgcagtgctgccataaccatgagtgataacactgcggccaacttacttctgacaacgatcggaggaccgaaggagctaaccgcttttttgcacaacatgggggatcatgtaactcgccttgatcgttgggaaccggagctgaatgaagccataccaaacgacgagcgtgacaccacgatgcctgcagcaatggcaacaacgttgcgcaaactattaactggcgaactacttactctagcttcccggcaacaattaatagactggatggaggcggataaagttgcaggaccacttctgcgctcggcccttccggctggctggtttattgctgataaatctggagccggtgagcgtgggtctcgcggtatcattgcagcactggggccagatggtaagccctcccgtatcgtagttatctacacgacggggagtcaggcaactatggatgaacgaaatagacagatcgctgagataggtgcctcactgattaagcattggtaactgtcagaccaagtttactcatatatactttagattgatttaaaacttcatttttaatttaaaaggatctaggtgaagatcctttttgataatctcatgaccaaaatcccttaacgtgagttttcgttccactgagcgtcagaccccgtagaaaagatcaaaggatcttcttgagatcctttttttctgcgcgtaatctgctgcttgcaaacaaaaaaaccaccgctaccagcggtggtttgtttgccggatcaagagctaccaactctttttccgaaggtaactggcttcagcagagcgcagataccaaatactgtccttctagtgtagccgtagttaggccaccacttcaagaactctgtagcaccgcctacatacctcgctctgctaatcctgttaccagtggctgctgccagtggcgataagtcgtgtcttaccgggttggactcaagacgatagttaccggataaggcgcagcggtcgggctgaacggggggttcgtgcacacagcccagcttggagcgaacgacctacaccgaactgagatacctacagcgtgagctatgagaaagcgccacgcttcccgaagggagaaaggcggacaggtatccggtaagcggcagggtcggaacaggagagcgcacgagggagcttccagggggaaacgcctggtatctttatagtcctgtcgggtttcgccacctctgacttgagcgtcgatttttgtgatgctcgtcaggggggcggagcctatggaaaaacgccagcaacgcggcctttttacggttcctggccttttgctggccttttgctcacatgttctttcctgcgttatcccctgattctgtggataaccgtattaccgcctttgagtgagctgataccgctcgccgcagccgaacgaccgagcgcagcgagtcagtgagcgaggaagcggaagagcgcctgatgcggtattttctccttacgcatctgtgcggtatttcacaccgcatatatggtgcactctcagtacaatctgctctgatgccgcatagttaagccagtatacactccgctatcgctacgtgactgggtcatggctgcgccccgacacccgccaacacccgctgacgcgccctgacgggcttgtctgctcccggcatccgcttacagacaagctgtgaccgtctccgggagctgcatgtgtcagaggttttcaccgtcatcaccgaaacgcgcgaggcagctgcggtaaagctcatcagcgtggtcgtgaagcgattcacagatgtctgcctgttcatccgcgtccagctcgttgagtttctccagaagcgttaatgtctggcttctgataaagcgggccatgttaagggcggttttttcctgtttggtcactgatgcctccgtgtaagggggatttctgttcatgggggtaatgataccgatgaaacgagagaggatgctcacgatacgggttactgatgatgaacatgcccggttactggaacgttgtgagggtaaacaactggcggtatggatgcggcgggaccagagaaaaatcactcagggtcaatgccagcgcttcgttaatacagatgtaggtgttccacagggtagccagcagcatcctgcgatgcagatccggaacataatggtgcagggcgctgacttccgcgtttccagactttacgaaacacggaaaccgaagaccattcatgttgttgctcaggtcgcagacgttttgcagcagcagtcgcttcacgttcgctcgcgtatcggtgattcattctgctaaccagtaaggcaaccccgccagcctagccgggtcctcaacgacaggagcacgatcatgcgcacccgtggccaggacccaacgctgcccgagatgcgccgcgtgcggctgctggagatggcggacgcgatggatatgttctgccaagggttggtttgcgcattcacagttctccgcaagaattgattggctccaattcttggagtggtgaatccgttagcgaggtgccgccggcttccattcaggtcgaggtggcccggctccatgcaccgcgacgcaacgcggggaggcagacaaggtatagggcggcgcctacaatccatgccaacccgttccatgtgctcgccgaggcggcataaatcgccgtgacgatcagcggtccagtgatcgaagttaggctggtaagagccgcgagcgatccttgaagctgtccctgatggtcgtcatctacctgcctggacagcatggcctgcaacgcgggcatcccgatgccgccggaagcgagaagaatcataatggggaaggccatccagcctcgcgtcgcgaacgccagcaagacgtagcccagcgcgtcggccgccatgccggcgataatggcctgcttctcgccgaaacgtttggtggcgggaccagtgacgaaggcttgagcgagggcgtgcaagattccgaataccgcaagcgacaggccgatcatcgtcgcgctccagcgaaagcggtcctcgccgaaaatgacccagagcgctgccggcacctgtcctacgagttgcatgataaagaagacagtcataagtgcggcgacgatagtcatgccccgcgcccaccggaaggagctgactgggttgaaggctctcaagggcatcggtcgagatcccggtgcctaatgagtgagctaacttacattaattgcgttgcgctcactgcccgctttccagtcgggaaacctgtcgtgccagctgcattaatgaatcggccaacgcgcggggagaggcggtttgcgtattgggcgccagggtggtttttcttttcaccagtgagacgggcaacagctgattgcccttcaccgcctggccctgagagagttgcagcaagcggtccacgctggtttgccccagcaggcgaaaatcctgtttgatggtggttaacggcgggatataacatgagctgtcttcggtatcgtcgtatcccactaccgagatatccgcaccaacgcgcagcccggactcggtaatggcgcgcattgcgcccagcgccatctgatcgttggcaaccagcatcgcagtgggaacgatgccctcattcagcatttgcatggtttgttgaaaaccggacatggcactccagtcgccttcccgttccgctatcggctgaatttgattgcgagtgagatatttatgccagccagccagacgcagacgcgccgagacagaacttaatgggcccgctaacagcgcgatttgctggtgacccaatgcgaccagatgctccacgcccagtcgcgtaccgtcttcatgggagaaaataatactgttgatgggtgtctggtcagagacatcaagaaataacgccggaacattagtgcaggcagcttccacagcaatggcatcctggtcatccagcggatagttaatgatcagcccactgacgcgttgcgcgagaagattgtgcaccgccgctttacaggcttcgacgccgcttcgttctaccatcgacaccaccacgctggcacccagttgatcggcgcgagatttaatcgccgcgacaatttgcgacggcgcgtgcagggccagactggaggtggcaacgccaatcagcaacgactgtttgcccgccagttgttgtgccacgcggttgggaatgtaattcagctccgccatcgccgcttccactttttcccgcgttttcgcagaaacgtggctggcctggttcaccacgcgggaaacggtctgataagagacaccggcatactctgcgacatcgtataacgttactggtttcacattcaccaccctgaattgactctcttccgggcgctatcatgccataccgcgaaaggttttgcgccattcgatggtgtccgggatctcgacgctctcccttatgcgactcctgcattaggaagc

SEQ ID NO: 12 - DNA, 2153 bp, synthetic construct
  source 1..2153: mol_type = other DNA
ggagtaatacgactcactatagggatccctatcagtgatagagaaatgcccacatactctgatgatccgagacggtcgggtccagatattcgtatctgtcgagtagagtgtgggctcggatcattcatggcaagagacggtcgggtccagatattcgtatctgtcgagtagagtgtgggctcttgccatgtgtatgtggggcttaatagcataaccccttggggcctctaaacgggtcttgaggggttttttgcgcttgttggagacgagctgcggccgcgattatcaaaaaggatcttcacctagatccttttaaattaaaaatgaagttttaaatcaatctaaagtatatatgagtaaacttggtctgacagttaccaatgcttaatcagtgaggcacctatctcagcgatctgtctatttcgttcatccatagttgcctgactccccgtcgtgtagataactacgatacgggagggcttaccatctggccccagtgctgcaatgataccgcgggacccacgctcaccggctccagatttatcagcaataaaccagccagccggaagggccgagcgcagaagtggtcctgcaactttatccgcctccatccagtctattaattgttgccgggaagctagagtaagtagttcgccagttaatagtttgcgcaacgttgttgccattgctacaggcatcgtggtgtcacgctcgtcgtttggtatggcttcattcagctccggttcccaacgatcaaggcgagttacatgatcccccatgttgtgcaaaaaagcggttagctccttcggtcctccgatcgttgtcagaagtaagttggccgcagtgttatcactcatggttatggcagcactgcataattctcttactgtcatgccatccgtaagatgcttttctgtgactggtgagtactcaaccaagtcattctgagaatagtgtatgcggcgaccgagttgctcttgcccggcgtcaatacgggataataccgcgccacatagcagaactttaaaagtgctcatcattggaaaacgttcttcggggcgaaaactctcaaggatcttaccgctgttgagatccagttcgatgtaacccactcgtgcacccaactgatcttcagcatcttttactttcaccagcgtttctgggtgagcaaaaacaggaaggcaaaatgccgcaaaaaagggaataagggcgacacggaaatgttgaatactcatactcttcctttttcaatattattgaagcatttatcagggttattgtctcatgagcggatacatatttgaatgtatttagaaaaataaacaaataggggttccgcgcacatttccccgaaaagtgccacctgtcatgaccaaaatcccttaacgtgagttttcgttccactgagcgtcagaccccgtagaaaagatcaaaggatcttcttgagatcctttttttctgcgcgtaatctgctgcttgcaaacaaaaaaaccaccgctaccagcggtggtttgtttgccggatcaagagctaccaactctttttccgaaggtaactggcttcagcagagcgcagataccaaatactgttcttctagtgtagccgtagttaggccaccacttcaagaactctgtagcaccgcctacatacctcgctctgctaatcctgttaccagtggctgctgccagtggcgataagtcgtgtcttaccgggttggactcaagacgatagttaccggataaggcgcagcggtcgggctgaacggggggttcgtgcacacagcccagcttggagcgaacgacctacaccgaactgagatacctacagcgtgagctatgagaaagcgccacgcttcccgaagggagaaaggcggacaggtatccggtaagcggcagggtcggaacaggagagcgcacgagggagcttccagggggaaacgcctggtatctttatagtcctgtcgggtttcgccacctctgacttgagcgtcgatttttgtgatgctcgtcaggggggcggagcctatggaaaaacgccagcaacgcggcctttttacggttcctggccttttgctggccttttgctcacatgttctttcctgcgttatcccctgattctgtggataaccgtgcggccgcaacacgtctcgagta

SEQ ID NO: 13 - DNA, 4804 bp, synthetic construct
  source 1..4804: mol_type = other DNA
agctgcggccgcgattatcaaaaaggatcttcacctagatccttttaaattaaaaatgaagttttaaatcaatctaaagtatatatgagtaaacttggtctgacagttaccaatgcttaatcagtgaggcacctatctcagcgatctgtctatttcgttcatccatagttgcctgactccccgtcgtgtagataactacgatacgggagggcttaccatctggccccagtgctgcaatgataccgcgggacccacgctcaccggctccagatttatcagcaataaaccagccagccggaagggccgagcgcagaagtggtcctgcaactttatccgcctccatccagtctattaattgttgccgggaagctagagtaagtagttcgccagttaatagtttgcgcaacgttgttgccattgctacaggcatcgtggtgtcacgctcgtcgtttggtatggcttcattcagctccggttcccaacgatcaaggcgagttacatgatcccccatgttgtgcaaaaaagcggttagctccttcggtcctccgatcgttgtcagaagtaagttggccgcagtgttatcactcatggttatggcagcactgcataattctcttactgtcatgccatccgtaagatgcttttctgtgactggtgagtactcaaccaagtcattctgagaatagtgtatgcggcgaccgagttgctcttgcccggcgtcaatacgggataataccgcgccacatagcagaactttaaaagtgctcatcattggaaaacgttcttcggggcgaaaactctcaaggatcttaccgctgttgagatccagttcgatgtaacccactcgtgcacccaactgatcttcagcatcttttactttcaccagcgtttctgggtgagcaaaaacaggaaggcaaaatgccgcaaaaaagggaataagggcgacacggaaatgttgaatactcatactcttcctttttcaatattattgaagcatttatcagggttattgtctcatgagcggatacatatttgaatgtatttagaaaaataaacaaataggggttccgcgcacatttccccgaaaagtgccacctgtcatgaccaaaatcccttaacgtgagttttcgttccactgagcgtcagaccccgtagaaaagatcaaaggatcttcttgagatcctttttttctgcgcgtaatctgctgcttgcaaacaaaaaaaccaccgctaccagcggtggtttgtttgccggatcaagagctaccaactctttttccgaaggtaactggcttcagcagagcgcagataccaaatactgttcttctagtgtagccgtagttaggccaccacttcaagaactctgtagcaccgcctacatacctcgctctgctaatcctgttaccagtggctgctgccagtggcgataagtcgtgtcttaccgggttggactcaagacgatagttaccggataaggcgcagcggtcgggctgaacggggggttcgtgcacacagcccagcttggagcgaacgacctacaccgaactgagatacctacagcgtgagctatgagaaagcgccacgcttcccgaagggagaaaggcggacaggtatccggtaagcggcagggtcggaacaggagagcgcacgagggagcttccagggggaaacgcctggtatctttatagtcctgtcgggtttcgccacctctgacttgagcgtcgatttttgtgatgctcgtcaggggggcggagcctatggaaaaacgccagcaacgcggcctttttacggttcctggccttttgctggccttttgctcacatgttctttcctgcgttatcccctgattctgtggataaccgtgcggccgcaacacgtctcgagtaggagtaatacgactcactatagtactagaccacaacggtttccctctagaaataattttgtttaactttaagaaggagatatacataatggttttcactttagaagacttcgtaggtgactggcgtcaaacagcaggttataatttagaccaagttttagaacaaggtggtgtatcaagtttattccaaaatttaggtgtttctgttactccaattcaacgtatcgtattaagtggtgaaaatggtcttaaaattgacatccatgttattattccttatgaaggtctttcaggtgaccaaatgggtcaaattgaaaaaatttttaaagtagtttatcctgtagatgaccatcactttaaagtaattttacactatggtactttagtaattgatggcgttacacctaatatgattgactactttggtcgtccttatgaaggtattgctgtttttgatggtaaaaaaatcacagttacaggtacattatggaatggtaataaaattattgacgaacgtttaatcaatcctgatggttcattattattccgtgttacaattaatggtgttacaggttggcgtctttgtgaacgtatccttgctgcttaaggtctcggcttaaataaataacggattgtgtccgtaatcacacgtggtgcgtacgataacgcatagtgtttttccctccacttaaatcgaagggttgtgtcttggatcgcgcgggtcaaatgtatatggttcatatacatccgcaggcacgtaataaagcgaggggttcgaatccccccgttacccccggtaggggcccacgcttgagaccactcatcgcgactagtagcggccgctgcagtccggcaaaaaagggcaaggtgtcaccaccctgccctttttctttaaaaccgaaaagattacttcgcgttatgcaggcttcctcgctcactgactcgctgcgctcggtcgttcggctgcggcgagcggtatcagctcactcaaaggcggtaatacggttatccacagaatcaggggataacgcaggaaagaacatgtgagcaaaaggccagcaaaaggccaggaaccgtaaaaaggccgcgttgctggcgtttttccacaggctccgcccccctgacgagcatcacaaaaatcgacgctcaagtcagaggtggcgaaacccgacaggactataaagataccaggcgtttccccctggaagctccctcgtgcgctctcctgttccgaccctgccgcttaccggatacctgtccgcctttctcccttcgggaagcgtggcgctttctcatagctcacgctgtaggtatctcagttcggtgtaggtcgttcgctccaagctgggctgtgtgcacgaaccccccgttcagcccgaccgctgcgccttatccggtaactatcgtcttgagtccaacccggtaagacacgacttatcgccactggcagcagccactggtaacaggattagcagagcgaggtatgtaggcggtgctacagagttcttgaagtggtggcctaactacggctacactagaagaacagtatttggtatctgcgctctgctgaagccagttaccttcggaaaaagagttggtagctcttgatccggcaaacaaaccaccgctggtagcggtggtttttttgtttgcaagcagcagattacgcgcagaaaaaaaggatctcaagaagatcctttgatcttttctacggggtctgacgctcagtggaacgaaaactcacgttaagggattttggtcatgagattatcaaaaaggatcttcacctagatccttttaaattaaaaatgaagttttaaatcaatctaaagtatatatgagtaaacttggtctgacagctcgaggcttggattctcaccaataaaaaacgcccggcggcaaccgagcgttctgaacaaatccagatggagttctgaggtcattactggatctatcaacaggagtccaagcgagctcgatatcaaattacgccccgccctgccactcatcgcagtactgttgtaattcattaagcattctgccgacatggaagccatcacaaacggcatgatgaacctgaatcgccagcggcatcagcaccttgtcgccttgcgtataatatttgcccatggtgaaaacgggggcgaagaagttgtccatattggccacgtttaaatcaaaactggtgaaactcacccagggattggctgaaacgaaaaacatattctcaataaaccctttagggaaataggccaggttttcaccgtaacacgccacatcttgcgaatatatgtgtagaaactgccggaaatcgtcgtggtattcactccagagcgatgaaaacgtttcagtttgctcatggaaaacggtgtaacaagggtgaacactatcccatatcaccagctcaccgtctttcattgccatacgaaattccggatgagcattcatcaggcgggcaagaatgtgaataaaggccggataaaacttgtgcttatttttctttacggtctttaaaaaggccgtaatatccagctgaacggtctggttataggtacattgagcaactgactgaaatgcctcaaaatgttctttacgatgccattgggatatatcaacggtggtatatccagtgatttttttctccattttagcttccttagctcctgaaaatctcgataactcaaaaaatacgcccggtagtgatcttatttcattatggtgaaagttggaacctcttacgtgcccgatcaactcgagtgccacctgacgtctaagaaaccattattatcatgacattaacctataaaaataggcgtatcacgaggcagaatttcagataaaaaaaatccttagctttcgctaaggatgatttctggaattcgcggccgcttctagagcgatgagtcgcttgttggagacg

SEQ ID NO: 14 - DNA, 978 bp, synthetic construct
  source 1..978: mol_type = other DNA
gcaccatcagccagaaaaccgaaccagccagaaaacgacctttctgtggatcttaaggctagagtactaatacgactcactatagggagaccacaacggtttccctctagaaataattttgtttaacttaagaaggaggaaaaaaaaatggtctctaaaggtgaagaattattcactggtgttgtcccaattttggttgaattagatggtgatgttaatggtcacaaattttctgtctccggtgaaggtgaaggtgatgctacttacggtaaattgaccttaaaatttatttgtactactggtaaattgccagttccatggccaaccttagtcactactttaacttatggtgttcaatgtttttctagatacccagatcatatgaaacaacatgactttttcaagtctgccatgccagaaggttatgttcaagaaagaactatttttttcaaagatgacggtaactacaagaccagagctgaagtcaagtttgaaggtgataccttagttaatagaatcgaattaaaaggtattgattttaaagaagatggtaacattttaggtcacaaattggaatacaactataactctcacaatgtttacatcatggctgacaaacaaaagaatggtatcaaagttaacttcaaaattagacacaacattgaagatggttctgttcaattagctgaccattatcaacaaaatactccaattggtgatggtccagtcttgttaccagacaaccattacttatccactcaatctgccttatccaaagatccaaacgaaaagagagaccacatggtcttgttagaatttgttactgctgctggtattaccttaggtatggatgaattgtacaaacaccaccatcatcaccactaataacgactcaggctgctacctagcataaccccttggggcctctaaacgggtcttgaggggttttttggcaggaaagaacatgtgagcaaaagg